European Patent Application EP 4 717 714 A1, published April 1, 2026. Title: 抗PD-1-抗VEGF的双特异性抗体、其药物组合物及其用途. Applicant: 上海君实生物医药科技股份有限公司. The sequence listing filed with the application follows.

SEQUENCE LISTING (34 sequences)

SEQ ID NO: 1 - protein, 5 aa, synthetic construct
DYEMH

SEQ ID NO: 2 - protein, 17 aa, synthetic construct
VIESETGGTAYNQKFKG

SEQ ID NO: 3 - protein, 16 aa, synthetic construct
EGITTVATTYYWYFDV

SEQ ID NO: 4 - protein, 16 aa, synthetic construct
RSSQSIVHSNGNTYLE

SEQ ID NO: 5 - protein, 7 aa, synthetic construct
KVSNRFS

SEQ ID NO: 6 - protein, 9 aa, synthetic construct
FQGSHVPLT

SEQ ID NO: 7 - protein, 5 aa, synthetic construct
ATDID

SEQ ID NO: 8 - protein, 17 aa, synthetic construct
RIFSPSDFTDYADSVKG

SEQ ID NO: 9 - protein, 20 aa, synthetic construct
PDTYAYNIFLDTPTYNALHY

SEQ ID NO: 10 - protein, 125 aa, synthetic construct [sequence omitted]

SEQ ID NO: 11 - protein, 112 aa, synthetic construct [sequence omitted]

SEQ ID NO: 12 - protein, 129 aa, synthetic construct
EVQLVESGGGLVQPGGSLRLSCAISGFSLAATDIDWVRQAPGKGLEWVARIFSPSDFTDYADSVKGRFTISADTSKNTVYLQMNSLRAEDTAVYYCGRPDTYAYNIFLDTPTYNALHYRGQGTLVTVSS

SEQ ID NO: 13 - protein, 219 aa, synthetic construct
DVVMTQSPLSLPVTLGQPASISCRSSQSIVHSNGNTYLEWYLQKPGQSPQLLIYKVSNRFSGVPDRFSGSGSGTDFTLKISRVEAEDVGVYYCFQGSHVPLTFGQGTKLEIKRTVAAPSVFIFPPSDEQLKSGTASVVCLLNNFYPREAKVQWKVDNALQSGNSQESVTEQDSKDSTYSLSSTLTLSKADYEKHKVYACEVTHQGLSSPVTKSFNRGEC

SEQ ID NO: 14 - protein, 596 aa, synthetic construct
EVQLVESGGGLVQPGGSLRLSCAISGFSLAATDIDWVRQAPGKGLEWVARIFSPSDFTDYADSVKGRFTISADTSKNTVYLQMNSLRAEDTAVYYCGRPDTYAYNIFLDTPTYNALHYRGQGTLVTVSSGGGGSGGGGSGGGGSQGQLVQSGAEVKKPGASVKVSCKASGYTFTDYEMHWVRQAPIHGLEWIGVIESETGGTAYNQKFKGRVTITADKSTSTAYMELSSLRSEDTAVYYCAREGITTVATTYYWYFDVWGQGTTVTVSSASTKGPSVFPLAPCSRSTSESTAALGCLVKDYFPEPVTVSWNSGALTSGVHTFPAVLQSSGLYSLSSVVTVPSSSLGTKTYTCNVDHKPSNTKVDKRVESKYGPPCPPCPAPEFLGGPSVFLFPPKPKDTLMISRTPEVTCVVVDVSQEDPEVQFNWYVDGVEVHNAKTKPREEQFNSTYRVVSVLTVLHQDWLNGKEYKCKVSNKGLPSSIEKTISKAKGQPREPQVYTLPPSQEEMTKNQVSLTCLVKGFYPSDIAVEWESNGQPENNYKTTPPVLDSDGSFFLYSRLTVDKSRWQEGNVFSCSVMHEALHNHYTQKSLSLSLGK

SEQ ID NO: 15 - protein, 594 aa, synthetic construct
QGQLVQSGAEVKKPGASVKVSCKASGYTFTDYEMHWVRQAPIHGLEWIGVIESETGGTAYNQKFKGRVTITADKSTSTAYMELSSLRSEDTAVYYCAREGITTVATTYYWYFDVWGQGTTVTVSSASTKGPSVFPLAPCSRSTSESTAALGCLVKDYFPEPVTVSWNSGALTSGVHTFPAVLQSSGLYSLSSVVTVPSSSLGTKTYTCNVDHKPSNTKVDKRVESKYGPPCPPCPAPEFLGGPSVFLFPPKPKDTLMISRTPEVTCVVVDVSQEDPEVQFNWYVDGVEVHNAKTKPREEQFNSTYRVVSVLTVLHQDWLNGKEYKCKVSNKGLPSSIEKTISKAKGQPREPQVYTLPPSQEEMTKNQVSLTCLVKGFYPSDIAVEWESNGQPENNYKTTPPVLDSDGSFFLYSRLTVDKSRWQEGNVFSCSVMHEALHNHYTQKSLSLSLGGGGSGGGGSGGGGSEVQLVESGGGLVQPGGSLRLSCAISGFSLAATDIDWVRQAPGKGLEWVARIFSPSDFTDYADSVKGRFTISADTSKNTVYLQMNSLRAEDTAVYYCGRPDTYAYNIFLDTPTYNALHYRGQGTLVTVSS

SEQ ID NO: 16 - protein, 601 aa, synthetic construct
QGQLVQSGAEVKKPGASVKVSCKASGYTFTDYEMHWVRQAPIHGLEWIGVIESETGGTAYNQKFKGRVTITADKSTSTAYMELSSLRSEDTAVYYCAREGITTVATTYYWYFDVWGQGTTVTVSSASTKGPSVFPLAPCSRSTSESTAALGCLVKDYFPEPVTVSWNSGALTSGVHTFPAVLQSSGLYSLSSVVTVPSSSLGTKTYTCNVDHKPSNTKVDKRVGGGGSGGGGSGGGGSEVQLVESGGGLVQPGGSLRLSCAISGFSLAATDIDWVRQAPGKGLEWVARIFSPSDFTDYADSVKGRFTISADTSKNTVYLQMNSLRAEDTAVYYCGRPDTYAYNIFLDTPTYNALHYRGQGTLVTVSSGGGGSESKYGPPCPPCPAPEFLGGPSVFLFPPKPKDTLMISRTPEVTCVVVDVSQEDPEVQFNWYVDGVEVHNAKTKPREEQFNSTYRVVSVLTVLHQDWLNGKEYKCKVSNKGLPSSIEKTISKAKGQPREPQVYTLPPSQEEMTKNQVSLTCLVKGFYPSDIAVEWESNGQPENNYKTTPPVLDSDGSFFLYSRLTVDKSRWQEGNVFSCSVMHEALHNHYTQKSLSLSLGK

SEQ ID NO: 17 - protein, 363 aa, synthetic construct
EVQLVESGGGLVQPGGSLRLSCAISGFSLAATDIDWVRQAPGKGLEWVARIFSPSDFTDYADSVKGRFTISADTSKNTVYLQMNSLRAEDTAVYYCGRPDTYAYNIFLDTPTYNALHYRGQGTLVTVSSGGGGSGGGGSGGGGSDVVMTQSPLSLPVTLGQPASISCRSSQSIVHSNGNTYLEWYLQKPGQSPQLLIYKVSNRFSGVPDRFSGSGSGTDFTLKISRVEAEDVGVYYCFQGSHVPLTFGQGTKLEIKRTVAAPSVFIFPPSDEQLKSGTASVVCLLNNFYPREAKVQWKVDNALQSGNSQESVTEQDSKDSTYSLSSTLTLSKADYEKHKVYACEVTHQGLSSPVTKSFNRGEC

SEQ ID NO: 18 - protein, 452 aa, synthetic construct
QGQLVQSGAEVKKPGASVKVSCKASGYTFTDYEMHWVRQAPIHGLEWIGVIESETGGTAYNQKFKGRVTITADKSTSTAYMELSSLRSEDTAVYYCAREGITTVATTYYWYFDVWGQGTTVTVSSASTKGPSVFPLAPCSRSTSESTAALGCLVKDYFPEPVTVSWNSGALTSGVHTFPAVLQSSGLYSLSSVVTVPSSSLGTKTYTCNVDHKPSNTKVDKRVESKYGPPCPPCPAPEFLGGPSVFLFPPKPKDTLMISRTPEVTCVVVDVSQEDPEVQFNWYVDGVEVHNAKTKPREEQFNSTYRVVSVLTVLHQDWLNGKEYKCKVSNKGLPSSIEKTISKAKGQPREPQVYTLPPSQEEMTKNQVSLTCLVKGFYPSDIAVEWESNGQPENNYKTTPPVLDSDGSFFLYSRLTVDKSRWQEGNVFSCSVMHEALHNHYTQKSLSLSLGK

SEQ ID NO: 19 - protein, 183 aa, synthetic construct
HHHHHHHHHHGGGSGGGSAPMAEGGGQNHHEVVKFMDVYQRSYCHPIETLVDIFQEYPDEIEYIFKPSCVPLMRCGGCCNDEGLECVPTEESNITMQIMRIKPHQGQHIGEMSFLQHNKCECRPKKDRARQENPCGPCSERRKHLFVQDPQTCKCSCKNTDSRCKARQLELNERTCRCDKPRR

SEQ ID NO: 20 - protein, 756 aa, synthetic construct
ASVGLPSVSLDLPRLSIQKDILTIKANTTLQITCRGQRDLDWLWPNNQSGSEQRVEVTECSDGLFCKTLTIPKVIGNDTGAYKCFYRETDLASVIYVYVQDYRSPFIASVSDQHGVVYITENKNKTVVIPCLGSISNLNVSLCARYPEKRFVPDGNRISWDSKKGFTIPSYMISYAGMVFCEAKINDESYQSIMYIVVVVGYRIYDVVLSPSHGIELSVGEKLVLNCTARTELNVGIDFNWEYPSSKHQHKKLVNRDLKTQSGSEMKKFLSTLTIDGVTRSDQGLYTCAASSGLMTKKNSTFVRVHEKPFVAFGSGMESLVEATVGERVRIPAKYLGYPPPEIKWYKNGIPLESNHTIKAGHVLTIMEVSERDTGNYTVILTNPISKEKQSHVVSLVVYVPPQIGEKSLISPVDSYQYGTTQTLTCTVYAIPPPHHIHWYWQLEEECANEPSQAVSVTNPYPCEEWRSVEDFQGGNKIEVNKNQFALIEGKNKTVSTLVIQAANVSALYKCEAVNKVGRGERVISFHVTRGPEITLQPDMQPTEQESVSLWCTADRSTFENLTWYKLGPQPLPIHVGELPTPVCKNLDTLWKLNATMFSNSTNDILIMELKNASLQDQGDYVCLAQDRKTKKRHCVVRQLTVLERVAPTITGNLENQTTSIGESIEVSCTASGNPPPQIMWFKDNETLVEDSGIVLKDGNRNLTIRRVRKEDEGLYTCQACSVLGCAKVEAFFIIEGAQEKTNLEAHHHHHHHHHH

SEQ ID NO: 21 - DNA, 336 bp, synthetic construct
  source 1..336: mol_type = other DNA
gatgtggtgatgacccagagcccgctgagcctgccggtgaccctgggccagccggcgagcattagctgccgcagcagccagagcattgtgcatagcaacggcaacacctatctggaatggtatctgcagaaaccgggccagagcccgcagctgctgatttataaagtgagcaaccgctttagcggcgtgccggatcgctttagcggcagcggcagcggcaccgattttaccctgaaaattagccgcgtggaagcggaagatgtgggcgtgtattattgctttcagggcagccatgtgccgctgacctttggccagggcaccaaactggaaattaaa

SEQ ID NO: 22 - DNA, 4792 bp, synthetic construct
  source 1..4792: mol_type = other DNA
gtacatttatattggctcatgtccaatatgaccgccatgttgacattgattattgactagttattaatagtaatcaattacggggtcattagttcatagcccatatatggagttccgcgttacataacttacggtaaatggcccgcctggctgaccgcccaacgacccccgcccattgacgtcaataatgacgtatgttcccatagtaacgccaatagggactttccattgacgtcaatgggtggagtatttacggtaaactgcccacttggcagtacatcaagtgtatcatatgccaagtccgccccctattgacgtcaatgacggtaaatggcccgcctggcattatgcccagtacatgaccttacgggactttcctacttggcagtacatctacgtattagtcatcgctattaccatggtgatgcggttttggcagtacaccaatgggcgtggatagcggtttgactcacggggatttccaagtctccaccccattgacgtcaatgggagtttgttttggcaccaaaatcaacgggactttccaaaatgtcgtaataaccccgccccgttgacgcaaatgggcggtaggcgtgtacggtgggaggtctatataagcagagctcgtttagtgaaccgtcagatcctcactctcttccgcatcgctgtctgcgagggccagctgttgggctcgcggttgaggacaaactcttcgcggtctttccagtactcttggatcggaaacccgtcggcctccgaacggtactccgccaccgagggacctgagcgagtccgcatcgaccggatcggaaaacctctcgagaaaggcgtctaaccagtcacagtcgcaaggtaggctgagcaccgtggcgggcggcagcgggtggcggtcggggttgtttctggcggaggtgctgctgatgatgtaattaaagtaggcggtcttgagacggcggatggtcgaggtgaggtgtggcaggcttgagatccagctgttggggtgagtactccctctcaaaagcgggcattacttctgcgctaagattgtcagtttccaaaaacgaggaggatttgatattcacctggcccgatctggccatacacttgagtgacaatgacatccactttgcctttctctccacaggtgtccactcccaggtccaagtttaaacggatctctagcgaattcgtcgactagaccaccatggacatgagggtgcccgctcagctcctggggctcctgctgctgtggctgagaggtgccagatgttgaagagcggatccgctcttctcgaactgtggctgcaccatctgtcttcatcttcccgccatctgatgagcagttgaaatctggaactgcctctgttgtgtgcctgctgaataacttctatcccagagaggccaaagtacagtggaaggtggataacgccctccaatcgggtaactcccaggagagtgtcacagagcaggacagcaaggacagcacctacagcctcagcagcaccctgacgctgagcaaagcagactacgagaaacacaaagtctacgcctgcgaagtcacccatcagggcctgagctcgcccgtcacaaagagcttcaacaggggagagtgttaggcggccgctcgaggccggcaaggccagatcccccgacctggacctctggctaataaaggaaatttattttcattgcaatagtgtgttggaattttttgtgtctctcactcggaaggacatatgggagggcaaatcatttggtcgagatccctcggagatctctagctagaggatcgatccccgccccggacgaactaaacctgactacgacatctctgccccttcttcgcggggcagtgcatgtaatcccttcagttggttggtacaacttgccaactgaaccctaaacgggtagcatatgcttcccgggtagtagtatatactatccagactaaccctaattcaatagcatatgttacccaacgggaagcatatgctatcgaattagggttagtaaaagggtcctaaggaacagcgatgtaggtgggcgggccaagataggggcgcgattgctgcgatctggaggacaaattacacacacttgcgcctgagcgccaagcacagggttgttggtcctcatattcacgaggtcgctgagagcacggtgggctaatgttgccatgggtagcatatactacccaaatatctggatagcatatgctatcctaatctatatctgggtagcataggctatcctaatctatatctgggtagcatatgctatcctaatctatatctgggtagtatatgctatcctaatttatatctgggtagcataggctatcctaatctatatctgggtagcatatgctatcctaatctatatctgggtagtatatgctatcctaatctgtatccgggtagcatatgctatcctaatagagattagggtagtatatgctatcctaatttatatctgggtagcatatactacccaaatatctggatagcatatgctatcctaatctatatctgggtagcatatgctatcctaatctatatctgggtagcataggctatcctaatctatatctgggtagcatatgctatcctaatctatatctgggtagtatatgctatcctaatttatatctgggtagcataggctatcctaatctatatctgggtagcatatgctatcctaatctatatctgggtagtatatgctatcctaatctgtatccgggtagcatatgctatcctcatgataagctgtcaaacatgagaattaattcttgaagacgaaagggcctcgtgatacgcctatttttataggttaatgtcatgataataatggtttcttagacgtcaggtggcacttttcggggaaatgtgcgcggaacccctatttgtttatttttctaaatacattcaaatatgtatccgctcatgagacaataaccctgataaatgcttcaataatattgaaaaaggaagagtatgagtattcaacatttccgtgtcgcccttattcccttttttgcggcattttgccttcctgtttttgctcacccagaaacgctggtgaaagtaaaagatgctgaagatcagttgggtgcacgagtgggttacatcgaactggatctcaacagcggtaagatccttgagagttttcgccccgaagaacgttttccaatgatgagcacttttaaagttctgctatgtggcgcggtattatcccgtgttgacgccgggcaagagcaactcggtcgccgcatacactattctcagaatgacttggttgagtactcaccagtcacagaaaagcatcttacggatggcatgacagtaagagaattatgcagtgctgccataaccatgagtgataacactgcggccaacttacttctgacaacgatcggaggaccgaaggagctaaccgcttttttgcacaacatgggggatcatgtaactcgccttgatcgttgggaaccggagctgaatgaagccataccaaacgacgagcgtgacaccacgatgcctgcagcaatggcaacaacgttgcgcaaactattaactggcgaactacttactctagcttcccggcaacaattaatagactggatggaggcggataaagttgcaggaccacttctgcgctcggcccttccggctggctggtttattgctgataaatctggagccggtgagcgtgggtctcgcggtatcattgcagcactggggccagatggtaagccctcccgtatcgtagttatctacacgacggggagtcaggcaactatggatgaacgaaatagacagatcgctgagataggtgcctcactgattaagcattggtaactgtcagaccaagtttactcatatatactttagattgatttaaaacttcatttttaatttaaaaggatctaggtgaagatcctttttgataatctcatgaccaaaatcccttaacgtgagttttcgttccactgagcgtcagaccccgtagaaaagatcaaaggatcttcttgagatcctttttttctgcgcgtaatctgctgcttgcaaacaaaaaaaccaccgctaccagcggtggtttgtttgccggatcaagagctaccaactctttttccgaaggtaactggcttcagcagagcgcagataccaaatactgttcttctagtgtagccgtagttaggccaccacttcaagaactctgtagcaccgcctacatacctcgctctgctaatcctgttaccagtggctgctgccagtggcgataagtcgtgtcttaccgggttggactcaagacgatagttaccggataaggcgcagcggtcgggctgaacggggggttcgtgcacacagcccagcttggagcgaacgacctacaccgaactgagatacctacagcgtgagctatgagaaagcgccacgcttcccgaagggagaaaggcggacaggtatccggtaagcggcagggtcggaacaggagagcgcacgagggagcttccagggggaaacgcctggtatctttatagtcctgtcgggtttcgccacctctgacttgagcgtcgatttttgtgatgctcgtcaggggggcggagcctatggaaaaacgccagcaacgcggcctttttacggttcctggccttttgctggccttttgctcacatgttctttcctgcgttatcccctgattctgtggataaccgtattaccgcctttgagtgagctgataccgctcgccgcagccgaacgaccgagcgcagcgagtcagtgagcgaggaagc

SEQ ID NO: 23 - DNA, 375 bp, synthetic construct
  source 1..375: mol_type = other DNA
cagggccagctggtgcagagcggcgccgaggtgaagaagcccggcgccagcgtgaaggtgagctgcaaggccagcggctacaccttcaccgactacgagatgcactgggtgagacaggcccccatccacggcctggagtggatcggcgtgatcgagagcgagaccggcggcaccgcctacaaccagaagttcaagggcagagtgaccatcaccgccgacaagagcaccagcaccgcctacatggagctgagcagcctgagaagcgaggacaccgccgtgtactactgcgccagagagggcatcaccaccgtggccaccacctactactggtacttcgacgtgtggggccagggcaccaccgtgaccgtgagcagc

SEQ ID NO: 24 - DNA, 5443 bp, synthetic construct
  source 1..5443: mol_type = other DNA
gtacatttatattggctcatgtccaatatgaccgccatgttgacattgattattgactagttattaatagtaatcaattacggggtcattagttcatagcccatatatggagttccgcgttacataacttacggtaaatggcccgcctggctgaccgcccaacgacccccgcccattgacgtcaataatgacgtatgttcccatagtaacgccaatagggactttccattgacgtcaatgggtggagtatttacggtaaactgcccacttggcagtacatcaagtgtatcatatgccaagtccgccccctattgacgtcaatgacggtaaatggcccgcctggcattatgcccagtacatgaccttacgggactttcctacttggcagtacatctacgtattagtcatcgctattaccatggtgatgcggttttggcagtacaccaatgggcgtggatagcggtttgactcacggggatttccaagtctccaccccattgacgtcaatgggagtttgttttggcaccaaaatcaacgggactttccaaaatgtcgtaataaccccgccccgttgacgcaaatgggcggtaggcgtgtacggtgggaggtctatataagcagagctcgtttagtgaaccgtcagatcctcactctcttccgcatcgctgtctgcgagggccagctgttgggctcgcggttgaggacaaactcttcgcggtctttccagtactcttggatcggaaacccgtcggcctccgaacggtactccgccaccgagggacctgagcgagtccgcatcgaccggatcggaaaacctctcgagaaaggcgtctaaccagtcacagtcgcaaggtaggctgagcaccgtggcgggcggcagcgggtggcggtcggggttgtttctggcggaggtgctgctgatgatgtaattaaagtaggcggtcttgagacggcggatggtcgaggtgaggtgtggcaggcttgagatccagctgttggggtgagtactccctctcaaaagcgggcattacttctgcgctaagattgtcagtttccaaaaacgaggaggatttgatattcacctggcccgatctggccatacacttgagtgacaatgacatccactttgcctttctctccacaggtgtccactcccaggtccaagtttaaacggatctctagcgaattcaagctttagaccaccatggaatggagctgggtgttcctgttctttctgtccgtgaccacaggcgtgcattcttgaagagcggatctgctcttctgctagcaccaagggccccagcgtgttccccctggccccttgcagcagaagcaccagcgagagcacagccgccctgggctgcctggtgaaggactacttccccgagcccgtgaccgtgtcctggaacagcggcgctctgaccagcggcgtgcataccttccccgccgtgctccagagcagcggactgtactccctgagcagcgtggtgaccgtgccttccagcagcctgggcaccaagacctacacctgcaacgtggaccacaagcccagcaacaccaaggtggacaagagagtggagagcaagtacggccctccctgccccccttgccctgcccccgagttcctgggcggacctagcgtgttcctgttcccccccaagcccaaggacaccctgatgatcagcagaacccccgaggtgacctgcgtggtggtggacgtgtcccaggaggaccccgaggtccagtttaattggtacgtggacggcgtggaagtgcataacgccaagaccaagcccagagaggagcagttcaacagcacctacagagtggtgtccgtgctgaccgtgctgcaccaggactggctgaacggcaaggaatacaagtgcaaggtctccaacaagggcctgcctagcagcatcgagaagaccatcagcaaggccaagggccagccacgggagccccaggtctacaccctgccacctagccaagaggagatgaccaagaaccaggtgtccctgacctgtctggtgaaaggcttctatcccagcgatatcgccgtggagtgggagagcaacggccagcccgagaacaactacaagaccaccccccctgtgctggacagcgacggcagcttcttcctgtactccagactgaccgtggacaagtccagatggcaggagggcaacgtcttcagctgctccgtgatgcacgaggccctgcacaaccactacacccagaagtccctgagcctgagcctgggcaagtgagcggccgctcgaggccggcaaggccagatcccccgacctggacctctggctaataaaggaaatttattttcattgcaatagtgtgttggaattttttgtgtctctcactcggaaggacatatgggagggcaaatcatttggtcgagatccctcggagatctctagctagaggatcgatccccgccccggacgaactaaacctgactacgacatctctgccccttcttcgcggggcagtgcatgtaatcccttcagttggttggtacaacttgccaactgaaccctaaacgggtagcatatgcttcccgggtagtagtatatactatccagactaaccctaattcaatagcatatgttacccaacgggaagcatatgctatcgaattagggttagtaaaagggtcctaaggaacagcgatgtaggtgggcgggccaagataggggcgcgattgctgcgatctggaggacaaattacacacacttgcgcctgagcgccaagcacagggttgttggtcctcatattcacgaggtcgctgagagcacggtgggctaatgttgccatgggtagcatatactacccaaatatctggatagcatatgctatcctaatctatatctgggtagcataggctatcctaatctatatctgggtagcatatgctatcctaatctatatctgggtagtatatgctatcctaatttatatctgggtagcataggctatcctaatctatatctgggtagcatatgctatcctaatctatatctgggtagtatatgctatcctaatctgtatccgggtagcatatgctatcctaatagagattagggtagtatatgctatcctaatttatatctgggtagcatatactacccaaatatctggatagcatatgctatcctaatctatatctgggtagcatatgctatcctaatctatatctgggtagcataggctatcctaatctatatctgggtagcatatgctatcctaatctatatctgggtagtatatgctatcctaatttatatctgggtagcataggctatcctaatctatatctgggtagcatatgctatcctaatctatatctgggtagtatatgctatcctaatctgtatccgggtagcatatgctatcctcatgataagctgtcaaacatgagaattaattcttgaagacgaaagggcctcgtgatacgcctatttttataggttaatgtcatgataataatggtttcttagacgtcaggtggcacttttcggggaaatgtgcgcggaacccctatttgtttatttttctaaatacattcaaatatgtatccgctcatgagacaataaccctgataaatgcttcaataatattgaaaaaggaagagtatgagtattcaacatttccgtgtcgcccttattcccttttttgcggcattttgccttcctgtttttgctcacccagaaacgctggtgaaagtaaaagatgctgaagatcagttgggtgcacgagtgggttacatcgaactggatctcaacagcggtaagatccttgagagttttcgccccgaagaacgttttccaatgatgagcacttttaaagttctgctatgtggcgcggtattatcccgtgttgacgccgggcaagagcaactcggtcgccgcatacactattctcagaatgacttggttgagtactcaccagtcacagaaaagcatcttacggatggcatgacagtaagagaattatgcagtgctgccataaccatgagtgataacactgcggccaacttacttctgacaacgatcggaggaccgaaggagctaaccgcttttttgcacaacatgggggatcatgtaactcgccttgatcgttgggaaccggagctgaatgaagccataccaaacgacgagcgtgacaccacgatgcctgcagcaatggcaacaacgttgcgcaaactattaactggcgaactacttactctagcttcccggcaacaattaatagactggatggaggcggataaagttgcaggaccacttctgcgctcggcccttccggctggctggtttattgctgataaatctggagccggtgagcgtgggtctcgcggtatcattgcagcactggggccagatggtaagccctcccgtatcgtagttatctacacgacggggagtcaggcaactatggatgaacgaaatagacagatcgctgagataggtgcctcactgattaagcattggtaactgtcagaccaagtttactcatatatactttagattgatttaaaacttcatttttaatttaaaaggatctaggtgaagatcctttttgataatctcatgaccaaaatcccttaacgtgagttttcgttccactgagcgtcagaccccgtagaaaagatcaaaggatcttcttgagatcctttttttctgcgcgtaatctgctgcttgcaaacaaaaaaaccaccgctaccagcggtggtttgtttgccggatcaagagctaccaactctttttccgaaggtaactggcttcagcagagcgcagataccaaatactgttcttctagtgtagccgtagttaggccaccacttcaagaactctgtagcaccgcctacatacctcgctctgctaatcctgttaccagtggctgctgccagtggcgataagtcgtgtcttaccgggttggactcaagacgatagttaccggataaggcgcagcggtcgggctgaacggggggttcgtgcacacagcccagcttggagcgaacgacctacaccgaactgagatacctacagcgtgagctatgagaaagcgccacgcttcccgaagggagaaaggcggacaggtatccggtaagcggcagggtcggaacaggagagcgcacgagggagcttccagggggaaacgcctggtatctttatagtcctgtcgggtttcgccacctctgacttgagcgtcgatttttgtgatgctcgtcaggggggcggagcctatggaaaaacgccagcaacgcggcctttttacggttcctggccttttgctggccttttgctcacatgttctttcctgcgttatcccctgattctgtggataaccgtattaccgcctttgagtgagctgataccgctcgccgcagccgaacgaccgagcgcagcgagtcagtgagcgaggaagc

SEQ ID NO: 25 - DNA, 727 bp, synthetic construct
  source 1..727: mol_type = other DNA
tgaagagcggatctgctcttctggcggaggcggatctgagagcaagtacggccctccctgccccccttgccctgcccccgagttcctgggcggacctagcgtgttcctgttcccccccaagcccaaggacaccctgatgatcagcagaacccccgaggtgacctgcgtggtggtggacgtgtcccaggaggaccccgaggtccagtttaattggtacgtggacggcgtggaagtgcataacgccaagaccaagcccagagaggagcagttcaacagcacctacagagtggtgtccgtgctgaccgtgctgcaccaggactggctgaacggcaaggaatacaagtgcaaggtctccaacaagggcctgcctagcagcatcgagaagaccatcagcaaggccaagggccagccacgggagccccaggtctacaccctgccacctagccaagaggagatgaccaagaaccaggtgtccctgacctgtctggtgaaaggcttctatcccagcgatatcgccgtggagtgggagagcaacggccagcccgagaacaactacaagaccaccccccctgtgctggacagcgacggcagcttcttcctgtactccagactgaccgtggacaagtccagatggcaggagggcaacgtcttcagctgctccgtgatgcacgaggccctgcacaaccactacacccagaagtccctgagcctgagcctgggcaagtga

SEQ ID NO: 26 - DNA, 387 bp, synthetic construct
  source 1..387: mol_type = other DNA
gaggtgcagctggtggagagcggaggcggactggtgcagcctggaggcagcctgagactgagctgcgccatcagcggattcagcctggccgccaccgacatcgactgggtgagacaggcccctggcaagggactggagtgggtggccagaatcttcagccccagcgacttcaccgactacgccgacagcgtgaagggcagattcaccatcagcgccgacaccagcaagaacaccgtgtacctgcagatgaacagcctgagagccgaggacaccgccgtgtactactgcggaagacctgacacctacgcctacaacatcttcctggacacccctacctacaacgccctgcactacagaggccagggaaccctggtgaccgtgagcagc

SEQ ID NO: 27 - DNA, 5179 bp, synthetic construct
  source 1..5179: mol_type = other DNA
gtacatttatattggctcatgtccaatatgaccgccatgttgacattgattattgactagttattaatagtaatcaattacggggtcattagttcatagcccatatatggagttccgcgttacataacttacggtaaatggcccgcctggctgaccgcccaacgacccccgcccattgacgtcaataatgacgtatgttcccatagtaacgccaatagggactttccattgacgtcaatgggtggagtatttacggtaaactgcccacttggcagtacatcaagtgtatcatatgccaagtccgccccctattgacgtcaatgacggtaaatggcccgcctggcattatgcccagtacatgaccttacgggactttcctacttggcagtacatctacgtattagtcatcgctattaccatggtgatgcggttttggcagtacaccaatgggcgtggatagcggtttgactcacggggatttccaagtctccaccccattgacgtcaatgggagtttgttttggcaccaaaatcaacgggactttccaaaatgtcgtaataaccccgccccgttgacgcaaatgggcggtaggcgtgtacggtgggaggtctatataagcagagctcgtttagtgaaccgtcagatcctcactctcttccgcatcgctgtctgcgagggccagctgttgggctcgcggttgaggacaaactcttcgcggtctttccagtactcttggatcggaaacccgtcggcctccgaacggtactccgccaccgagggacctgagcgagtccgcatcgaccggatcggaaaacctctcgagaaaggcgtctaaccagtcacagtcgcaaggtaggctgagcaccgtggcgggcggcagcgggtggcggtcggggttgtttctggcggaggtgctgctgatgatgtaattaaagtaggcggtcttgagacggcggatggtcgaggtgaggtgtggcaggcttgagatccagctgttggggtgagtactccctctcaaaagcgggcattacttctgcgctaagattgtcagtttccaaaaacgaggaggatttgatattcacctggcccgatctggccatacacttgagtgacaatgacatccactttgcctttctctccacaggtgtccactcccaggtccaagtttaaacggatctctagcgaattcgtcgactagaccaccatggacatgagggtgcccgctcagctcctggggctcctgctgctgtggctgagaggtgccagatgttgaagagcggatctgctcttctgctagcggcggaggcggatctgagagcaagtacggccctccctgccccccttgccctgcccccgagttcctgggcggacctagcgtgttcctgttcccccccaagcccaaggacaccctgatgatcagcagaacccccgaggtgacctgcgtggtggtggacgtgtcccaggaggaccccgaggtccagtttaattggtacgtggacggcgtggaagtgcataacgccaagaccaagcccagagaggagcagttcaacagcacctacagagtggtgtccgtgctgaccgtgctgcaccaggactggctgaacggcaaggaatacaagtgcaaggtctccaacaagggcctgcctagcagcatcgagaagaccatcagcaaggccaagggccagccacgggagccccaggtctacaccctgccacctagccaagaggagatgaccaagaaccaggtgtccctgacctgtctggtgaaaggcttctatcccagcgatatcgccgtggagtgggagagcaacggccagcccgagaacaactacaagaccaccccccctgtgctggacagcgacggcagcttcttcctgtactccagactgaccgtggacaagtccagatggcaggagggcaacgtcttcagctgctccgtgatgcacgaggccctgcacaaccactacacccagaagtccctgagcctgagcctgggcaagtgagcggccgctcgaggccggcaaggccagatcccccgacctcgacctctggctaataaaggaaatttattttcattgcaatagtgtgttggaattttttgtgtctctcactcggaaggacatatgggagggcaaatcatttggtcgagatccctcggagatctctagctagaggatcgatccccgccccggacgaactaaacctgactacgacatctctgccccttcttcgcggggcagtgcatgtaatcccttcagttggttggtacaacttgccaactgaaccctaaacgggtagcatatgcttcccgggtagtagtatatactatccagactaaccctaattcaatagcatatgttacccaacgggaagcatatgctatcgaattagggttagtaaaagggtcctaaggaacagcgatgtaggtgggcgggccaagataggggcgcgattgctgcgatctggaggacaaattacacacacttgcgcctgagcgccaagcacagggttgttggtcctcatattcacgaggtcgctgagagcacggtgggctaatgttgccatgggtagcatatactacccaaatatctggatagcatatgctatcctaatctatatctgggtagcataggctatcctaatctatatctgggtagcatatgctatcctaatctatatctgggtagtatatgctatcctaatttatatctgggtagcataggctatcctaatctatatctgggtagcatatgctatcctaatctatatctgggtagtatatgctatcctaatctgtatccgggtagcatatgctatcctaatagagattagggtagtatatgctatcctaatttatatctgggtagcatatactacccaaatatctggatagcatatgctatcctaatctatatctgggtagcatatgctatcctaatctatatctgggtagcataggctatcctaatctatatctgggtagcatatgctatcctaatctatatctgggtagtatatgctatcctaatttatatctgggtagcataggctatcctaatctatatctgggtagcatatgctatcctaatctatatctgggtagtatatgctatcctaatctgtatccgggtagcatatgctatcctcatgataagctgtcaaacatgagaattaattcttgaagacgaaagggcctcgtgatacgcctatttttataggttaatgtcatgataataatggtttcttagacgtcaggtggcacttttcggggaaatgtgcgcggaacccctatttgtttatttttctaaatacattcaaatatgtatccgctcatgagacaataaccctgataaatgcttcaataatattgaaaaaggaagagtatgagtattcaacatttccgtgtcgcccttattcccttttttgcggcattttgccttcctgtttttgctcacccagaaacgctggtgaaagtaaaagatgctgaagatcagttgggtgcacgagtgggttacatcgaactggatctcaacagcggtaagatccttgagagttttcgccccgaagaacgttttccaatgatgagcacttttaaagttctgctatgtggcgcggtattatcccgtgttgacgccgggcaagagcaactcggtcgccgcatacactattctcagaatgacttggttgagtactcaccagtcacagaaaagcatcttacggatggcatgacagtaagagaattatgcagtgctgccataaccatgagtgataacactgcggccaacttacttctgacaacgatcggaggaccgaaggagctaaccgcttttttgcacaacatgggggatcatgtaactcgccttgatcgttgggaaccggagctgaatgaagccataccaaacgacgagcgtgacaccacgatgcctgcagcaatggcaacaacgttgcgcaaactattaactggcgaactacttactctagcttcccggcaacaattaatagactggatggaggcggataaagttgcaggaccacttctgcgctcggcccttccggctggctggtttattgctgataaatctggagccggtgagcgtgggtctcgcggtatcattgcagcactggggccagatggtaagccctcccgtatcgtagttatctacacgacggggagtcaggcaactatggatgaacgaaatagacagatcgctgagataggtgcctcactgattaagcattggtaactgtcagaccaagtttactcatatatactttagattgatttaaaacttcatttttaatttaaaaggatctaggtgaagatcctttttgataatctcatgaccaaaatcccttaacgtgagttttcgttccactgagcgtcagaccccgtagaaaagatcaaaggatcttcttgagatcctttttttctgcgcgtaatctgctgcttgcaaacaaaaaaaccaccgctaccagcggtggtttgtttgccggatcaagagctaccaactctttttccgaaggtaactggcttcagcagagcgcagataccaaatactgttcttctagtgtagccgtagttaggccaccacttcaagaactctgtagcaccgcctacatacctcgctctgctaatcctgttaccagtggctgctgccagtggcgataagtcgtgtcttaccgggttggactcaagacgatagttaccggataaggcgcagcggtcgggctgaacggggggttcgtgcacacagcccagcttggagcgaacgacctacaccgaactgagatacctacagcgtgagctatgagaaagcgccacgcttcccgaagggagaaaggcggacaggtatccggtaagcggcagggtcggaacaggagagcgcacgagggagcttccagggggaaacgcctggtatctttatagtcctgtcgggtttcgccacctctgacttgagcgtcgatttttgtgatgctcgtcaggggggcggagcctatggaaaaacgccagcaacgcggcctttttacggttcctggccttttgctggccttttgctcacatgttctttcctgcgttatcccctgattctgtggataaccgtattaccgcctttgagtgagctgataccgctcgccgcagccgaacgaccgagcgcagcgagtcagtgagcgaggaagc

SEQ ID NO: 28 - DNA, 807 bp, synthetic construct
  source 1..807: mol_type = other DNA
gaggtgcagctggtggagagcggaggcggactggtgcagcctggaggcagcctgagactgagctgcgccatcagcggattcagcctggccgccaccgacatcgactgggtgagacaggcccctggcaagggactggagtgggtggccagaatcttcagccccagcgacttcaccgactacgccgacagcgtgaagggcagattcaccatcagcgccgacaccagcaagaacaccgtgtacctgcagatgaacagcctgagagccgaggacaccgccgtgtactactgcggaagacctgacacctacgcctacaacatcttcctggacacccctacctacaacgccctgcactacagaggccagggaaccctggtgaccgtgagcagcggaggcggaggctccggaggcggaggcagcggaggcggaggatcccagggccagctggtgcagagcggcgccgaggtgaagaagcccggcgccagcgtgaaggtgagctgcaaggccagcggctacaccttcaccgactacgagatgcactgggtgagacaggcccccatccacggcctggagtggatcggcgtgatcgagagcgagaccggcggcaccgcctacaaccagaagttcaagggcagagtgaccatcaccgccgacaagagcaccagcaccgcctacatggagctgagcagcctgagaagcgaggacaccgccgtgtactactgcgccagagagggcatcaccaccgtggccaccacctactactggtacttcgacgtgtggggccagggcaccaccgtgaccgtgagcagc

SEQ ID NO: 29 - DNA, 1418 bp, synthetic construct
  source 1..1418: mol_type = other DNA
gctagcaccaagggccccagcgtgttccccctggccccttgcagcagaagcaccagcgagagcacagccgccctgggctgcctggtgaaggactacttccccgagcccgtgaccgtgtcctggaacagcggcgctctgaccagcggcgtgcataccttccccgccgtgctccagagcagcggactgtactccctgagcagcgtggtgaccgtgccttccagcagcctgggcaccaagacctacacctgcaacgtggaccacaagcccagcaacaccaaggtggacaagagagtggagagcaagtacggccctccctgccccccttgccctgcccccgagttcctgggcggacctagcgtgttcctgttcccccccaagcccaaggacaccctgatgatcagcagaacccccgaggtgacctgcgtggtggtggacgtgtcccaggaggaccccgaggtccagtttaattggtacgtggacggcgtggaagtgcataacgccaagaccaagcccagagaggagcagttcaacagcacctacagagtggtgtccgtgctgaccgtgctgcaccaggactggctgaacggcaaggaatacaagtgcaaggtctccaacaagggcctgcctagcagcatcgagaagaccatcagcaaggccaagggccagccacgggagccccaggtctacaccctgccacctagccaagaggagatgaccaagaaccaggtgtccctgacctgtctggtgaaaggcttctatcccagcgatatcgccgtggagtgggagagcaacggccagcccgagaacaactacaagaccaccccccctgtgctggacagcgacggcagcttcttcctgtactccagactgaccgtggacaagtccagatggcaggagggcaacgtcttcagctgctccgtgatgcacgaggccctgcacaaccactacacccagaagtccctgagcctgagcctgggaggcggaggatccggaggcggaggcagcggaggcggaggcagcgaggtgcagctggtggagagcggaggcggactggtgcagcctggaggcagcctgagactgagctgcgccatcagcggattcagcctggccgccaccgacatcgactgggtgagacaggcccctggcaagggactggagtgggtggccagaatcttcagccccagcgacttcaccgactacgccgacagcgtgaagggcagattcaccatcagcgccgacaccagcaagaacaccgtgtacctgcagatgaacagcctgagagccgaggacaccgccgtgtactactgcggaagacctgacacctacgcctacaacatcttcctggacacccctacctacaacgccctgcactacagaggccagggaaccctggtgaccgtgagcagctgagcggccgc

SEQ ID NO: 30 - DNA, 1116 bp, synthetic construct
  source 1..1116: mol_type = other DNA
cagggccagctggtgcagagcggcgccgaggtgaagaagcccggcgccagcgtgaaggtgagctgcaaggccagcggctacaccttcaccgactacgagatgcactgggtgagacaggcccccatccacggcctggagtggatcggcgtgatcgagagcgagaccggcggcaccgcctacaaccagaagttcaagggcagagtgaccatcaccgccgacaagagcaccagcaccgcctacatggagctgagcagcctgagaagcgaggacaccgccgtgtactactgcgccagagagggcatcaccaccgtggccaccacctactactggtacttcgacgtgtggggccagggcaccaccgtgaccgtgagcagcgctagcaccaagggccccagcgtgttccccctggccccttgcagcagaagcaccagcgagagcacagccgccctgggctgcctggtgaaggactacttccccgagcccgtgaccgtgtcctggaacagcggcgctctgaccagcggcgtgcataccttccccgccgtgctccagagcagcggactgtactccctgagcagcgtggtgaccgtgccttccagcagcctgggcaccaagacctacacctgcaacgtggaccacaagcccagcaacaccaaggtggacaagagagtgggaggcggaggctccggaggcggaggcagcggaggcggaggatccgaggtgcagctggtggagagcggaggcggactggtgcagcctggaggcagcctgagactgagctgcgccatcagcggattcagcctggccgccaccgacatcgactgggtgagacaggcccctggcaagggactggagtgggtggccagaatcttcagccccagcgacttcaccgactacgccgacagcgtgaagggcagattcaccatcagcgccgacaccagcaagaacaccgtgtacctgcagatgaacagcctgagagccgaggacaccgccgtgtactactgcggaagacctgacacctacgcctacaacatcttcctggacacccctacctacaacgccctgcactacagaggccagggaaccctggtgaccgtgagcagcggcggaggcggatct

SEQ ID NO: 31 - protein, 219 aa, synthetic construct; identical to SEQ ID NO: 13

SEQ ID NO: 32 - protein, 452 aa, synthetic construct; identical to SEQ ID NO: 18

SEQ ID NO: 33 - protein, 363 aa, synthetic construct
EVQLVESGGGLVQPGGSLRLSCAISGFSLAATDIDWVRQAPGKGLEWVARIFSPSDFTDYADSVKGRFTISADTSKNTVYLQMNSLRAEDTAVYYCGRPDTYAYNIFLDTPTYNALHYRGQGTLVTVSSGGGGSESKYGPPCPPCPAPEFLGGPSVFLFPPKPKDTLMISRTPEVTCVVVDVSQEDPEVQFNWYVDGVEVHNAKTKPREEQFNSTYRVVSVLTVLHQDWLNGKEYKCKVSNKGLPSSIEKTISKAKGQPREPQVYTLPPSQEEMTKNQVSLTCLVKGFYPSDIAVEWESNGQPENNYKTTPPVLDSDGSFFLYSRLTVDKSRWQEGNVFSCSVMHEALHNHYTQKSLSLSLGK

SEQ ID NO: 34 - DNA, 1092 bp, synthetic construct
  source 1..1092: mol_type = other DNA
gaggtgcagctggtggagagcggaggcggactggtgcagcctggaggcagcctgagactgagctgcgccatcagcggattcagcctggccgccaccgacatcgactgggtgagacaggcccctggcaagggactggagtgggtggccagaatcttcagccccagcgacttcaccgactacgccgacagcgtgaagggcagattcaccatcagcgccgacaccagcaagaacaccgtgtacctgcagatgaacagcctgagagccgaggacaccgccgtgtactactgcggaagacctgacacctacgcctacaacatcttcctggacacccctacctacaacgccctgcactacagaggccagggaaccctggtgaccgtgagcagcggaggcggaggctccggaggcggaggcagcggaggcggaggatccgatgtggtgatgacccagagcccgctgagcctgccggtgaccctgggccagccggcgagcattagctgccgcagcagccagagcattgtgcatagcaacggcaacacctatctggaatggtatctgcagaaaccgggccagagcccgcagctgctgatttataaagtgagcaaccgctttagcggcgtgccggatcgctttagcggcagcggcagcggcaccgattttaccctgaaaattagccgcgtggaagcggaagatgtgggcgtgtattattgctttcagggcagccatgtgccgctgacctttggccagggcaccaaactggaaattaaacgaactgtggctgcaccatctgtcttcatcttcccgccatctgatgagcagttgaaatctggaactgcctctgttgtgtgcctgctgaataacttctatcccagagaggccaaagtacagtggaaggtggataacgccctccaatcgggtaactcccaggagagtgtcacagagcaggacagcaaggacagcacctacagcctcagcagcaccctgacgctgagcaaagcagactacgagaaacacaaagtctacgcctgcgaagtcacccatcagggcctgagctcgcccgtcacaaagagcttcaacaggggagagtgttag